European Patent Application EP 4 553 158 A1, published May 14, 2025. Title: HSL PROTEIN, GENE, VECTOR, CELL, COMPOSITION AND USE THEREOF, AND METHOD FOR IMPROVING HERBICIDE RESISTANCE OF CROPS. Applicant: Central China Normal University. The sequence listing filed with the application follows.

SEQUENCE LISTING (4 sequences)

SEQ ID NO: 1 - protein, 350 aa, Oryza sativa
MADESWRTPAIVQELAAAGVEEPPSRYVLGEKDRSDELVAAELPEPIPVVDLSRLAGADEAAKLRAALQNWGFFLLTNHGVETSLMDDVLNLAREFFNQPIERKRKFSNLIDGKNFQVEGYGTDRVVTQDQILDWSDRLFLRVEPKEERNLAFWPDHPESFRDVLNEYASRTKRIRDDIVQAMSKLLGLDEDYFFDRLNKAPALARFNYYPPCPRPDLVFGVRPHSDGSLFTILLVDEDVGGLQIQRDGKWYNVQVTPNTLLINLGDTMEVLCNGIFRSPVHRVVTNAERERISLAMFYSVNDEKDIGPAAGLLDENRPARYRKVSVGEFRAGIIGKFSRRERYIDSLKI

SEQ ID NO: 2 - protein, 351 aa, Oryza sativa
MADESWRAPAIVQELAAAGVEEPPSRYLLREKDRSDVKLVAAELPEPLPVVDLSRLDGAEEATKLRVALQNWGFFLLTNHGVEASLMDSVMNLSREFFNQPIERKQKFSNLIDGKNFQIQGYGTDRVVTQDQILDWSDRLHLRVEPKEEQDLAFWPDHPESFRDVLNKYASGTKRIRDDIIQAMAKLLELDEDYFLDRLNEAPAFARFNYYPPCPRPDLVFGIRPHSDGTLLTILLVDKDVSGLQVQRDGKWSNVEATPHTLLINLGDTMEVMCNGIFRSPVHRVVTNAEKERISLAMLYSVNDEKDIEPAAGLLDENRPARYRKVSVEEFRAGIFGKFSRGERYIDSLRI

SEQ ID NO: 3 - DNA, 1053 bp, Oryza sativa
  source 1..1053: mol_type = genomic DNA
atggctgacgagtcatggaggacgccggcgatagtgcaagagctggcggcggccggcgtcgaggagccaccgagtcggtacgtgcttggggagaaagaccgttctgacgagctggtcgccgccgagctgccggagcccatccccgtcgttgatctcagccggctagccggcgccgacgaggctgccaagctcagggcggctctgcagaattggggcttcttcctgcttaccaaccatggagtagaaacctctctgatggatgatgtgttgaacttggcaagagagttcttcaaccaaccgatcgaacggaagcgaaaattcagcaacttgatcgacggcaagaacttccaggtggaagggtatggaactgaccgggtggtaacccaagatcagatcctggactggtctgatcggctgtttctcagagttgaacccaaggaggagcgaaatcttgccttctggcctgaccatcctgaatctttcagggatgttctgaacgagtacgcatcaagaaccaaaagaataagagacgatatcgttcaggctatgtccaagcttcttgggcttgatgaggattacttcttcgaccgactcaacaaagctcctgcacttgcaagattcaactactaccctccctgtccaaggcctgaccttgtgttcggcgtcaggcctcactccgacggctccctctttacgattcttctcgtcgacgaagatgtcggtggcctgcaaattcagagggatggcaagtggtacaatgttcaggtcactcccaacacattgctgatcaacttaggtgacaccatggaggtattgtgcaatggcatcttcaggagcccagtgcacagggtggtgacaaacgccgagagggagaggatctcactggccatgttttacagtgtgaatgatgagaaagatattgggccggcggctggtttgctggatgagaatcggcctgcaagatacaggaaagtgagcgtcggagagttcagggctgggatcattggaaaattctctcgacgagagagatacatcgactccctgaagatctga

SEQ ID NO: 4 - DNA, 1056 bp, Oryza sativa
  source 1..1056: mol_type = genomic DNA
atggctgacgagtcatggagggcgccggcgatagtgcaagagctggcggcagccggcgtcgaggagccgccgagccgatacctgctacgggagaaagaccgttctgacgtcaagctggtcgccgccgagctgccggagcccctccccgtcgttgatctcagccggctagatggtgccgaggaggccaccaagctcagggtggctctgcagaattggggcttcttcctgcttaccaaccatggagtagaagcctctctgatggacagcgtgatgaacttgtcgagagagtttttcaaccaaccaatcgaacggaagcaaaaattcagcaacttgatcgatggcaagaacttccagattcaagggtatggaactgaccgggtggttacccaagatcagatcctggactggtctgatcggttgcatctcagagttgaacccaaggaggagcaagatcttgccttctggcctgaccatcctgaatctttcagggatgttctgaacaagtatgcatcaggaaccaaaagaattagagacgatatcattcaggctatggccaagcttcttgagcttgatgaggattacttcttggaccgactcaacgaagctcctgcatttgcaagattcaactactaccctccctgtccaaggcctgaccttgtgttcggcatcaggcctcactccgacggcaccctcttgacgattcttctcgtcgacaaagatgtcagtggcctgcaagttcagagggatggcaagtggtccaacgttgaggcaactcctcacacattgctgatcaacttaggtgacaccatggaggtaatgtgcaatggcatcttcaggagcccggtgcacagggtggtgacaaacgccgagaaggagaggatctccctggccatgttatacagcgtgaacgatgagaaagacattgagccggcggctggtttgctggatgagaatcggcctgcaagatacaggaaagtgagcgtcgaagagttcagggccgggatctttggaaaattctctcgaggagagaggtacatcgactccctgaggatctga